European Patent Application EP 4 534 550 A1, published April 9, 2025. Title: NCgl2747 Gene Mutant and Use Thereof in Preparation of L-lysine. Applicant: Ningxia Eppen Biotech Co., Ltd. Application CN. The sequence listing filed with the application follows.

SEQUENCE LISTING (38 sequences)

SEQ ID NO: 1 - DNA, 1314 bp, Corynebacterium glutamicum
  source 1..1314: mol_type = unassigned DNA
gtgactacagacaagcgcaaaacctctaagaccaccgacaccgccaacaaggctgtgggcgcggatcaggcagcgcgtcccactcggcgaacaactcgccgcatcttcgatcagtcggagaagatgaaggacgtgctgtacgagatccgtggcccggtggccgcggaggcggaacgcatggagcttgatgggcataacatcttaaagctcaacacgggaaatccagccgtgttcggattcgatgcccccgacgtgattatgcgtgacatgatcgccaaccttccaacttcccaagggtattccacctccaaaggcattattccggcccggcgagcagtggtcacccgctacgaagttgtgcccggattcccccacttcgatgttgatgatgtgttcttaggcaacggtgtctcagaactaatcaccatgaccacccaagcactcctcaacgacggcgatgaagttcttatccccgcaccggactacccactgtggactgccgcaacctccctggctggtggtaagcctgtgcactacctctgtgatgaggaagatgactggaacccatccatcgaagacatcaagtccaaaatctcagagaaaaccaaagctattgtggtgatcaaccccaacaaccccacgggagctgtctacccgcgccgggtgttggaacaaatcgtcgagattgcacgcgagcatgacctgctgattttggccgatgaaatctacgaccgcattctctacgatgatgccgagcacatcagcctggcaacccttgcaccagatctcctttgcatcacatacaacggtctatccaaggcataccgcgtcgcaggataccgagctggctggatggtattgactggaccaaagcaatacgcacgtggatttattgagggcctcgaactcctcgcaggcactcgactctgcccaaatgtcccagctcagcacgctattcaggtagctctcggtggacgccagtccatctacgacctcactggcgaacacggccgactcctggaacagcgcaacatggcatggacgaaactcaacgaaatcccaggtgtcagctgtgtgaaaccaatgggagctctatacgcgttccccaagctcgaccccaacgtgtacgaaatccacgacgacacccaactcatgctggatcttctccgtgccgagaaaatcctcatggttcagggcactggcttcaactggccacatcacgatcacttccgagtggtcaccctgccatgggcatcccagttggaaaacgcaattgagcgcctgggtaacttcctgtccacttacaagcagtag

SEQ ID NO: 2 - protein, 437 aa, Corynebacterium glutamicum
MTTDKRKTSKTTDTANKAVGADQAARPTRRTTRRIFDQSEKMKDVLYEIRGPVAAEAERMELDGHNILKLNTGNPAVFGFDAPDVIMRDMIANLPTSQGYSTSKGIIPARRAVVTRYEVVPGFPHFDVDDVFLGNGVSELITMTTQALLNDGDEVLIPAPDYPLWTAATSLAGGKPVHYLCDEEDDWNPSIEDIKSKISEKTKAIVVINPNNPTGAVYPRRVLEQIVEIAREHDLLILADEIYDRILYDDAEHISLATLAPDLLCITYNGLSKAYRVAGYRAGWMVLTGPKQYARGFIEGLELLAGTRLCPNVPAQHAIQVALGGRQSIYDLTGEHGRLLEQRNMAWTKLNEIPGVSCVKPMGALYAFPKLDPNVYEIHDDTQLMLDLLRAEKILMVQGTGFNWPHHDHFRVVTLPWASQLENAIERLGNFLSTYKQ

SEQ ID NO: 3 - DNA, 1314 bp, Artificial sequence
  source 1..1314: mol_type = other DNA
gtgactacagacaagcgcaaaacctctaagaccaccgacaccgccaacaaggctgtgggcgcggatcaggcagcgcgtcccactcggcgaacaactcgccgcatcttcgatcagtcggagaagatgaaggacgtgctgtacgagatccgtggcccggtggccgcggaggcggaacgcatggagcttgatgggcataacatcttaaagctcaacacgggaaatccagccgtgttcggattcgatgcccccgacgtgattatgcgtgacatgatcgccaaccttccaacttcccaagggtattccacctccaaaggcattattccggcccggcgagcagtggtcacccgctacgaagttgtgcccggattcccccacttcgatgttgatgatgtgttcttaggcaacggtgtctcagaactaatcaccatgaccacccaagcactcctcaacgacggcgatgaagttcttatccccgcaccggactacccactgtggactgccgcaacctccctggctggtggtaagcctgtgcactacctctgtgatgaggaagatgactggaacccatccatcgaagacatcaagtccaaaatctcagagaaaaccaaagctattgtggtgatcaaccccaacaaccccacgggagctgtctacccgcgccgggtgttggaacaaatcgtcgagattgcacgcgagcatgacctgctgattttggccgatgaaatctacgaccgcattctctacgatgatgccgagcacatcagcctggcaacccttgcaccagatctcctttgcatcacatacaacggtctatccaaggcataccgcgtcgcaggataccgagctggctggatggtattgactggaccaaagcaatacgcacgtggatttattgagggcctcgaactcctcgcaggcactcgactctgcccaaatgtcccagctcagcacgcttttcaggtagctctcggtggacgccagtccatctacgacctcactggcgaacacggccgactcctggaacagcgcaacatggcatggacgaaactcaacgaaatcccaggtgtcagctgtgtgaaaccaatgggagctctatacgcgttccccaagctcgaccccaacgtgtacgaaatccacgacgacacccaactcatgctggatcttctccgtgccgagaaaatcctcatggttcagggcactggcttcaactggccacatcacgatcacttccgagtggtcaccctgccatgggcatcccagttggaaaacgcaattgagcgcctgggtaacttcctgtccacttacaagcagtag

SEQ ID NO: 4 - protein, 437 aa, Artificial sequence
MTTDKRKTSKTTDTANKAVGADQAARPTRRTTRRIFDQSEKMKDVLYEIRGPVAAEAERMELDGHNILKLNTGNPAVFGFDAPDVIMRDMIANLPTSQGYSTSKGIIPARRAVVTRYEVVPGFPHFDVDDVFLGNGVSELITMTTQALLNDGDEVLIPAPDYPLWTAATSLAGGKPVHYLCDEEDDWNPSIEDIKSKISEKTKAIVVINPNNPTGAVYPRRVLEQIVEIAREHDLLILADEIYDRILYDDAEHISLATLAPDLLCITYNGLSKAYRVAGYRAGWMVLTGPKQYARGFIEGLELLAGTRLCPNVPAQHAFQVALGGRQSIYDLTGEHGRLLEQRNMAWTKLNEIPGVSCVKPMGALYAFPKLDPNVYEIHDDTQLMLDLLRAEKILMVQGTGFNWPHHDHFRVVTLPWASQLENAIERLGNFLSTYKQ

SEQ ID NO: 5 - DNA, 1296 bp, Artificial sequence
  source 1..1296: mol_type = other DNA
tcacccgctacgaagttgtgcccggattcccccacttcgatgttgatgatgtgttcttaggcaacggtgtctcagaactaatcaccatgaccacccaagcactcctcaacgacggcgatgaagttcttatccccgcaccggactacccactgtggactgccgcaacctccctggctggtggtaagcctgtgcactacctctgtgatgaggaagatgactggaacccatccatcgaagacatcaagtccaaaatctcagagaaaaccaaagctattgtggtgatcaaccccaacaaccccacgggagctgtctacccgcgccgggtgttggaacaaatcgtcgagattgcacgcgagcatgacctgctgattttggccgatgaaatctacgaccgcattctctacgatgatgccgagcacatcagcctggcaacccttgcaccagatctcctttgcatcacatacaacggtctatccaaggcataccgcgtcgcaggataccgagctggctggatggtattgactggaccaaagcaatacgcacgtggatttattgagggcctcgaactcctcgcaggcactcgactctgcccaaatgtcccagctcagcacgcttttcaggtagctctcggtggacgccagtccatctacgacctcactggcgaacacggccgactcctggaacagcgcaacatggcatggacgaaactcaacgaaatcccaggtgtcagctgtgtgaaaccaatgggagctctatacgcgttccccaagctcgaccccaacgtgtacgaaatccacgacgacacccaactcatgctggatcttctccgtgccgagaaaatcctcatggttcagggcactggcttcaactggccacatcacgatcacttccgagtggtcaccctgccatgggcatcccagttggaaaacgcaattgagcgcctgggtaacttcctgtccacttacaagcagtagtagttgttaggattcaccacgaatctcaggatttttgagattcgtggtgaatttttgcgttttccagtcaggctcctgcaactttcggaccgatttcagaggggcggagctggtttgtggtggatccttgaaatggaacctcgcaggaagctttcaggaagaccaagttgggcctaggggtggcgggattgcaaaaatccgtccccggttcgccatgaaatgctgattttgatcgaatctttgcgctaactgtagggcgggttcagggggtgaatgcaccacgagcaacccgaagggtgcgaagtgggcattcgtagaacaa

SEQ ID NO: 6 - DNA, 763 bp, Artificial sequence
  source 1..763: mol_type = other DNA
aatgcgttctggactgaggtgaccaccatgcaagacgaggtggacctagtgatcaccaacccgccgttttctctgttccgtgagttcctgagttggctattacacggtgacgtgttgttttctatcatcggtaacgcgaacgtaatcacatatctaggtgcctgaatctagattaaaactataaacattatttaaaaccattgccttattggagcatgctgcaagcttttcgcggtgggcttgcaacatcttacatcagaatgaatgatgttaaacacctaataagttcaagtagttaaaaggaaatatcaacaatgttacgaaaagcatctatcacgctaatgatatccgttacgctcttaacatgtgcctctccagcacaggcactgtcatcacaagcactctcgtcagaaagctccacttcgcagagtgattctcctacgcaatttgttgcgagtatagctgcgcccttcaataagaacttaacctatgagcagcgcaaagccattcgtttcggacctacgacagaacaagaagcagaacaatgcttggcaaagtatggtcgcgatggcgaggggccatggcctgctattgctatctatcctgactgctccttcgatactatcgaacaagatttctatgatcaagcaatatccaaagccctctcagtaatcagtctgggaagctcctagaagactcgtaacgaccaaaagcaccgagaacagatgcaactcaagcccatttacatctgttctcggtgcac

SEQ ID NO: 7 - DNA, 1645 bp, Artificial sequence
  source 1..1645: mol_type = other DNA
caaagcacttgctactcaatcatggtaaacagcctggtcgcagtccttcacgattcaaactttgccttccgctacgccttccacctgatcatcatagaagacggtgaagtaacagcagccggagatcccacagagatcgtcactgcgggactgatcgaagaagtctacaacgtcaaagcctgtgcatcccagaccccgtgaacagcaaaccgatgatcgtgccactggaaagatcttaggcagccgtgggattacacccttttagagctagaacagtaaaaattcacccaatagctttcaactacgcacacaaagtggcaacattgagcgggtgactacagacaagcgcaaaacctctaagaccaccgacaccgccaacaaggctgtgggcgcggatcaggcagcgcgtcccactcggcgaacaactcgccgcatcttcgatcagtcggagaagatgaaggacgtgctgtacgagatccgtggcccggtggccgcggaggcggaacgcatggagcttgatgggcataacatcttaaagctcaacacgggaaatccagccgtgttcggattcgatgcccccgacgtgattatgcgtgacatgatcgccaaccttccaacttcccaagggtattccacctccaaaggcattattccggcccggcgagcagtggtcacccgctacgaagttgtgcccggattcccccacttcgatgttgatgatgtgttcttaggcaacggtgtctcagaactaatcaccatgaccacccaagcactcctcaacgacggcgatgaagttcttatccccgcaccggactacccactgtggactgccgcaacctccctggctggtggtaagcctgtgcactacctctgtgatgaggaagatgactggaacccatccatcgaagacatcaagtccaaaatctcagagaaaaccaaagctattgtggtgatcaaccccaacaaccccacgggagctgtctacccgcgccgggtgttggaacaaatcgtcgagattgcacgcgagcatgacctgctgattttggccgatgaaatctacgaccgcattctctacgatgatgccgagcacatcagcctggcaacccttgcaccagatctcctttgcatcacatacaacggtctatccaaggcataccgcgtcgcaggataccgagctggctggatggtattgactggaccaaagcaatacgcacgtggatttattgagggcctcgaactcctcgcaggcactcgactctgcccaaatgtcccagctcagcacgctattcaggtagctctcggtggacgccagtccatctacgacctcactggcgaacacggccgactcctggaacagcgcaacatggcatggacgaaactcaacgaaatcccaggtgtcagctgtgtgaaaccaatgggagctctatacgcgttccccaagctcgaccccaacgtgtacgaaatccacgacgacacccaactcatgctggatcttctccgtgccgagaaaatcctcatggttcagggcactggcttcaactggccacatcacgatcacttccgagtggtcaccctgccatgggcatcccagttggaaaacgcaattgagcgcctgggtaacttcctgtccacttacaagcagtag

SEQ ID NO: 8 - DNA, 1645 bp, Artificial sequence
  source 1..1645: mol_type = other DNA
caaagcacttgctactcaatcatggtaaacagcctggtcgcagtccttcacgattcaaactttgccttccgctacgccttccacctgatcatcatagaagacggtgaagtaacagcagccggagatcccacagagatcgtcactgcgggactgatcgaagaagtctacaacgtcaaagcctgtgcatcccagaccccgtgaacagcaaaccgatgatcgtgccactggaaagatcttaggcagccgtgggattacacccttttagagctagaacagtaaaaattcacccaatagctttcaactacgcacacaaagtggcaacattgagcgggtgactacagacaagcgcaaaacctctaagaccaccgacaccgccaacaaggctgtgggcgcggatcaggcagcgcgtcccactcggcgaacaactcgccgcatcttcgatcagtcggagaagatgaaggacgtgctgtacgagatccgtggcccggtggccgcggaggcggaacgcatggagcttgatgggcataacatcttaaagctcaacacgggaaatccagccgtgttcggattcgatgcccccgacgtgattatgcgtgacatgatcgccaaccttccaacttcccaagggtattccacctccaaaggcattattccggcccggcgagcagtggtcacccgctacgaagttgtgcccggattcccccacttcgatgttgatgatgtgttcttaggcaacggtgtctcagaactaatcaccatgaccacccaagcactcctcaacgacggcgatgaagttcttatccccgcaccggactacccactgtggactgccgcaacctccctggctggtggtaagcctgtgcactacctctgtgatgaggaagatgactggaacccatccatcgaagacatcaagtccaaaatctcagagaaaaccaaagctattgtggtgatcaaccccaacaaccccacgggagctgtctacccgcgccgggtgttggaacaaatcgtcgagattgcacgcgagcatgacctgctgattttggccgatgaaatctacgaccgcattctctacgatgatgccgagcacatcagcctggcaacccttgcaccagatctcctttgcatcacatacaacggtctatccaaggcataccgcgtcgcaggataccgagctggctggatggtattgactggaccaaagcaatacgcacgtggatttattgagggcctcgaactcctcgcaggcactcgactctgcccaaatgtcccagctcagcacgcttttcaggtagctctcggtggacgccagtccatctacgacctcactggcgaacacggccgactcctggaacagcgcaacatggcatggacgaaactcaacgaaatcccaggtgtcagctgtgtgaaaccaatgggagctctatacgcgttccccaagctcgaccccaacgtgtacgaaatccacgacgacacccaactcatgctggatcttctccgtgccgagaaaatcctcatggttcagggcactggcttcaactggccacatcacgatcacttccgagtggtcaccctgccatgggcatcccagttggaaaacgcaattgagcgcctgggtaacttcctgtccacttacaagcagtag

SEQ ID NO: 9 - DNA, 596 bp, Artificial sequence
  source 1..596: mol_type = other DNA
cagatggcgcaattaaatcaagatctcagaactcatttttcaatctcttcttttagggcacccgtcatcaattgagctatcggccattcattaaaaactgcgcgtcgatcaaccgaaagctgagtaagcaaaaaattcgcctcttctctatcgtcaagaagcaaagcgcaaccaatcataatctcgctatagttgtctgggtgcattgtttgatcaagattatgcctaaaagatcgaatttctgttctttgtgaatccagtaatccagtttggcgatacaaaatttgccaaccattaagcctgtaaattggcgactcttctcgatctcgttccacgagccaatcattgagagcttgagctgctataagaaatgcagttttcctgctctgctcagaatcagctgccttaattaggcgaagcaccatccatgtggcgagattatcaacatcaacagtttcttcaagcgctgaatagaaatcaacaagcttatccaaatgcagattcaatactgatggaagccatcgattatcaatgagctcgtacggcgtcactcgctcgattgaggagtcgctccgatccgttgaaggtgtcatagc

SEQ ID NO: 10 - DNA, 1959 bp, Artificial sequence
  source 1..1959: mol_type = other DNA
tccaaggaagatacacgcccgaagaagctccgttaatggacgctcttctattaagccttttctgatggatacaagcagagaatcagtcatgctaaatatcataatccatcaaacatttgatcggtgtcaatcaatgcgttctggactgaggtgaccaccatgcaagacgaggtggacctagtgatcaccaacccgccgttttctctgttccgtgagttcctgagttggctattacacggtgacgtgttgttttctatcatcggtaacgcgaacgtaatcacatatctaggtgcctgaatctagattaaaactataaacattatttaaaaccattgccttattggagcatgctgcaagcttttcgcggtgggcttgcaacatcttacatcagaatgaatgatgttaaacacctaataagttcaagtagttaaaaggaaatatcaacaatgttacgaaaagcatctatcacgctaatgatatccgttacgctcttaacatgtgcctctccagcacaggcactgtcatcacaagcactctcgtcagaaagctccacttcgcagagtgattctcctacgcaatttgttgcgagtatagctgcgcccttcaataagaacttaacctatgagcagcgcaaagccattcgtttcggacctacgacagaacaagaagcagaacaatgcttggcaaagtatggtcgcgatggcgaggggccatggcctgctattgctatctatcctgactgctccttcgatactatcgaacaagatttctatgatcaagcaatatccaaagccctctcagtaatcagtctgggaagctcctagaagactcgtaacgaccaaaagcaccgagaacagatgcaactcaagcccatttacatctgttctcggtgcaccaaagcacttgctactcaatcatggtaaacagcctggtcgcagtccttcacgattcaaactttgccttccgctacgccttccacctgatcatcatagaagacggtgaagtaacagcagccggagatcccacagagatcgtcactgcgggactgatcgaagaagtctacaacgtcaaagcctgtgcatcccagaccccgtgaacagcaaaccgatgatcgtgccactggaaagatcttaggcagccgtgggattacacccttttagagctagaacagtaaaaattcacccaatagctttcaactacgcacacaaagtggcaacattgagcgggtgactacagacaagcgcaaaacctctaagaccaccgacaccgccaacaaggctgtgggcgcggatcaggcagcgcgtcccactcggcgaacaactcgccgcatcttcgatcagtcggagaagatgaaggacgtgctgtacgagatccgtggcccggtggccgcggaggcggaacgcatggagcttgatgggcataacatcttaaagctcaacacgggaaatccagccgtgttcggattcgatgcccccgacgtgattatgcgtgacatgatcgccaaccttccaacttcccaagggtattccacctccaaaggcattattccggcccggcgagcagtggtcacccgctacgaagttgtgcccggattcccccacttcgatgttgatgatgtgttcttaggcaacggtgtctcagaactaatcaccatgaccacccaagcactcctcaacgacggcgatgaagttcttatccccgcaccggactacccactgtggactgccgcaacctccctggctggtggtaagcctgtgcactacctctgtgatgaggaagatgactggaacccatccatcgaagacatcaagtccaaaatctcagagaaaaccaaagctattgtggtgatcaaccccaacaaccccacgggagctgtctacccgcgccgggtgttggaacaaatcgtcgagattgcacgcgagcatgacctgctgattttggccgatgaaatctacgacc

SEQ ID NO: 11 - DNA, 1600 bp, Artificial sequence
  source 1..1600: mol_type = other DNA
caacggtgtctcagaactaatcaccatgaccacccaagcactcctcaacgacggcgatgaagttcttatccccgcaccggactacccactgtggactgccgcaacctccctggctggtggtaagcctgtgcactacctctgtgatgaggaagatgactggaacccatccatcgaagacatcaagtccaaaatctcagagaaaaccaaagctattgtggtgatcaaccccaacaaccccacgggagctgtctacccgcgccgggtgttggaacaaatcgtcgagattgcacgcgagcatgacctgctgattttggccgatgaaatctacgaccgcattctctacgatgatgccgagcacatcagcctggcaacccttgcaccagatctcctttgcatcacatacaacggtctatccaaggcataccgcgtcgcaggataccgagctggctggatggtattgactggaccaaagcaatacgcacgtggatttattgagggcctcgaactcctcgcaggcactcgactctgcccaaatgtcccagctcagcacgctattcaggtagctctcggtggacgccagtccatctacgacctcactggcgaacacggccgactcctggaacagcgcaacatggcatggacgaaactcaacgaaatcccaggtgtcagctgtgtgaaaccaatgggagctctatacgcgttccccaagctcgaccccaacgtgtacgaaatccacgacgacacccaactcatgctggatcttctccgtgccgagaaaatcctcatggttcagggcactggcttcaactggccacatcacgatcacttccgagtggtcaccctgccatgggcatcccagttggaaaacgcaattgagcgcctgggtaacttcctgtccacttacaagcagtagcagatggcgcaattaaatcaagatctcagaactcatttttcaatctcttcttttagggcacccgtcatcaattgagctatcggccattcattaaaaactgcgcgtcgatcaaccgaaagctgagtaagcaaaaaattcgcctcttctctatcgtcaagaagcaaagcgcaaccaatcataatctcgctatagttgtctgggtgcattgtttgatcaagattatgcctaaaagatcgaatttctgttctttgtgaatccagtaatccagtttggcgatacaaaatttgccaaccattaagcctgtaaattggcgactcttctcgatctcgttccacgagccaatcattgagagcttgagctgctataagaaatgcagttttcctgctctgctcagaatcagctgccttaattaggcgaagcaccatccatgtggcgagattatcaacatcaacagtttcttcaagcgctgaatagaaatcaacaagcttatccaaatgcagattcaatactgatggaagccatcgattatcaatgagctcgtacggcgtcactcgctcgattgaggagtcgctccgatccgttgaaggtgtcatagcaaaatgatgacgcttggaaattacttcatgataagtccactcccctgcaacatcaccagggtgagctatcaacgcaagattccaacgacca

SEQ ID NO: 12 - DNA, 1715 bp, Artificial sequence
  source 1..1715: mol_type = other DNA
gcttgcatgcctgcaggtcgactctagaggatcccccaaagcacttgctactcaatcatggtaaacagcctggtcgcagtccttcacgattcaaactttgccttccgctacgccttccacctgatcatcatagaagacggtgaagtaacagcagccggagatcccacagagatcgtcactgcgggactgatcgaagaagtctacaacgtcaaagcctgtgcatcccagaccccgtgaacagcaaaccgatgatcgtgccactggaaagatcttaggcagccgtgggattacacccttttagagctagaacagtaaaaattcacccaatagctttcaactacgcacacaaagtggcaacattgagcgggtgactacagacaagcgcaaaacctctaagaccaccgacaccgccaacaaggctgtgggcgcggatcaggcagcgcgtcccactcggcgaacaactcgccgcatcttcgatcagtcggagaagatgaaggacgtgctgtacgagatccgtggcccggtggccgcggaggcggaacgcatggagcttgatgggcataacatcttaaagctcaacacgggaaatccagccgtgttcggattcgatgcccccgacgtgattatgcgtgacatgatcgccaaccttccaacttcccaagggtattccacctccaaaggcattattccggcccggcgagcagtggtcacccgctacgaagttgtgcccggattcccccacttcgatgttgatgatgtgttcttaggcaacggtgtctcagaactaatcaccatgaccacccaagcactcctcaacgacggcgatgaagttcttatccccgcaccggactacccactgtggactgccgcaacctccctggctggtggtaagcctgtgcactacctctgtgatgaggaagatgactggaacccatccatcgaagacatcaagtccaaaatctcagagaaaaccaaagctattgtggtgatcaaccccaacaaccccacgggagctgtctacccgcgccgggtgttggaacaaatcgtcgagattgcacgcgagcatgacctgctgattttggccgatgaaatctacgaccgcattctctacgatgatgccgagcacatcagcctggcaacccttgcaccagatctcctttgcatcacatacaacggtctatccaaggcataccgcgtcgcaggataccgagctggctggatggtattgactggaccaaagcaatacgcacgtggatttattgagggcctcgaactcctcgcaggcactcgactctgcccaaatgtcccagctcagcacgctattcaggtagctctcggtggacgccagtccatctacgacctcactggcgaacacggccgactcctggaacagcgcaacatggcatggacgaaactcaacgaaatcccaggtgtcagctgtgtgaaaccaatgggagctctatacgcgttccccaagctcgaccccaacgtgtacgaaatccacgacgacacccaactcatgctggatcttctccgtgccgagaaaatcctcatggttcagggcactggcttcaactggccacatcacgatcacttccgagtggtcaccctgccatgggcatcccagttggaaaacgcaattgagcgcctgggtaacttcctgtccacttacaagcagtaggttttggcggatgagagaagattttcagcctgat

SEQ ID NO: 13 - DNA, 1715 bp, Artificial sequence
  source 1..1715: mol_type = other DNA
gcttgcatgcctgcaggtcgactctagaggatcccccaaagcacttgctactcaatcatggtaaacagcctggtcgcagtccttcacgattcaaactttgccttccgctacgccttccacctgatcatcatagaagacggtgaagtaacagcagccggagatcccacagagatcgtcactgcgggactgatcgaagaagtctacaacgtcaaagcctgtgcatcccagaccccgtgaacagcaaaccgatgatcgtgccactggaaagatcttaggcagccgtgggattacacccttttagagctagaacagtaaaaattcacccaatagctttcaactacgcacacaaagtggcaacattgagcgggtgactacagacaagcgcaaaacctctaagaccaccgacaccgccaacaaggctgtgggcgcggatcaggcagcgcgtcccactcggcgaacaactcgccgcatcttcgatcagtcggagaagatgaaggacgtgctgtacgagatccgtggcccggtggccgcggaggcggaacgcatggagcttgatgggcataacatcttaaagctcaacacgggaaatccagccgtgttcggattcgatgcccccgacgtgattatgcgtgacatgatcgccaaccttccaacttcccaagggtattccacctccaaaggcattattccggcccggcgagcagtggtcacccgctacgaagttgtgcccggattcccccacttcgatgttgatgatgtgttcttaggcaacggtgtctcagaactaatcaccatgaccacccaagcactcctcaacgacggcgatgaagttcttatccccgcaccggactacccactgtggactgccgcaacctccctggctggtggtaagcctgtgcactacctctgtgatgaggaagatgactggaacccatccatcgaagacatcaagtccaaaatctcagagaaaaccaaagctattgtggtgatcaaccccaacaaccccacgggagctgtctacccgcgccgggtgttggaacaaatcgtcgagattgcacgcgagcatgacctgctgattttggccgatgaaatctacgaccgcattctctacgatgatgccgagcacatcagcctggcaacccttgcaccagatctcctttgcatcacatacaacggtctatccaaggcataccgcgtcgcaggataccgagctggctggatggtattgactggaccaaagcaatacgcacgtggatttattgagggcctcgaactcctcgcaggcactcgactctgcccaaatgtcccagctcagcacgcttttcaggtagctctcggtggacgccagtccatctacgacctcactggcgaacacggccgactcctggaacagcgcaacatggcatggacgaaactcaacgaaatcccaggtgtcagctgtgtgaaaccaatgggagctctatacgcgttccccaagctcgaccccaacgtgtacgaaatccacgacgacacccaactcatgctggatcttctccgtgccgagaaaatcctcatggttcagggcactggcttcaactggccacatcacgatcacttccgagtggtcaccctgccatgggcatcccagttggaaaacgcaattgagcgcctgggtaacttcctgtccacttacaagcagtaggttttggcggatgagagaagattttcagcctgat

SEQ ID NO: 14 - DNA, 1400 bp, Artificial sequence
  source 1..1400: mol_type = other DNA
gcagcaagtagcctgggtattcgccacggacgtgaatattgccgaaggcatagtcctcgtgggacttttgctgggcggtaagttgatcgcgtgggtccggggtaatgccataacgaggaacggcaataatcatgcaaccgatctggttttgtgggtcgatctcatgagcaatcttagttgccaaagcacttgctactcaatcatggtaaacagcctggtcgcagtccttcacgattcaaactttgccttccgctacgccttccacctgatcatcatagaagacggtgaagtaacagcagccggagatcccacagagatcgtcactgcgggactgatcgaagaagtctacaacgtcaaagcctgtgcatcccagaccccgtgaacagcaaaccgatgatcgtgccactggaaagatcttaggcagccgtgggattacacccttttagagctagaacagtaaaaattcacccaatagctttcaactacgcacacaaagtggcaacattgagcgggtgactacagacaagcgcaaaacctctaagaccaccgacaccgccaacaaggctgtgggcgcggatcaggcagcgcgtcccactcggcgaacaactcgccgcatcttcgatcagtcggagaagatgaaggacgtgggtaacttcctgtccacttacaagcagtagtagttgttaggattcaccacgaatctcaggatttttgagattcgtggtgaatttttgcgttttccagtcaggctcctgcaactttcggaccgatttcagaggggcggagctggtttgtggtggatccttgaaatggaacctcgcaggaagctttcaggaagaccaagttgggcctaggggtggcgggattgcaaaaatccgtccccggttcgccatgaaatgctgattttgatcgaatctttgcgctaactgtagggcgggttcagggggtgaatgcaccacgagcaacccgaagggtgcgaagtgggcattcgtagaacaatcccagaggaaagccgtacggctttcctcgacatgatcaatcaaggtatgtcaggtcttgctgcgtctacagcggtcggggtcagtgaattcaccgggcgaaagtgggcgaaggccgccggggtgaaactgacccgcggcccgcgaggtggcaatgcttttgacaccgccgagaaacttgagattgcagccagcatgctagagaaaggatgcctaccccgagaaatcggcgagtatgtcggcatgactcgggccaatatatccctatggcgcaaacaaggcccagacaagcttcgccaacgcgcagccaccttgcgcaccggcaagcgagcagctgaattcatccacgccccggtgatgggcccttattatgggccacgcacactccatcaagtgttgcgt

SEQ ID NO: 15 - DNA, 55 bp, synthetic construct
  source 1..55: mol_type = other DNA
cagtgccaagcttgcatgcctgcaggtcgactctagtcacccgctacgaagttgt

SEQ ID NO: 16 - DNA, 33 bp, synthetic construct
  source 1..33: mol_type = other DNA
ctacctgaaaagcgtgctgagctgggacatttg

SEQ ID NO: 17 - DNA, 42 bp, synthetic construct
  source 1..42: mol_type = other DNA
caaatgtcccagctcagcacgcttttcaggtagctctcggtg

SEQ ID NO: 18 - DNA, 57 bp, synthetic construct
  source 1..57: mol_type = other DNA
cagctatgaccatgattacgaattcgagctcggtacccttgttctacgaatgcccac

SEQ ID NO: 19 - DNA, 18 bp, synthetic construct
  source 1..18: mol_type = other DNA
tgtaaaacgacggccagt

SEQ ID NO: 20 - DNA, 18 bp, synthetic construct
  source 1..18: mol_type = other DNA
caggaaacagctatgacc

SEQ ID NO: 21 - DNA, 19 bp, synthetic construct
  source 1..19: mol_type = other DNA
tctatccaaggcataccgc

SEQ ID NO: 22 - DNA, 19 bp, synthetic construct
  source 1..19: mol_type = other DNA
tcccattggtttcacacag

SEQ ID NO: 23 - DNA, 55 bp, synthetic construct
  source 1..55: mol_type = other DNA
cagtgccaagcttgcatgcctgcaggtcgactctagaatgcgttctggactgagg

SEQ ID NO: 24 - DNA, 39 bp, synthetic construct
  source 1..39: mol_type = other DNA
gattgagtagcaagtgctttggtgcaccgagaacagatg

SEQ ID NO: 25 - DNA, 39 bp, synthetic construct
  source 1..39: mol_type = other DNA
catctgttctcggtgcaccaaagcacttgctactcaatc

SEQ ID NO: 26 - DNA, 41 bp, synthetic construct
  source 1..41: mol_type = other DNA
gatttaattgcgccatctgctactgcttgtaagtggacagg

SEQ ID NO: 27 - DNA, 41 bp, synthetic construct
  source 1..41: mol_type = other DNA
cctgtccacttacaagcagtagcagatggcgcaattaaatc

SEQ ID NO: 28 - DNA, 60 bp, synthetic construct
  source 1..60: mol_type = other DNA
cagctatgaccatgattacgaattcgagctcggtacccgctatgacaccttcaacggatc

SEQ ID NO: 29 - DNA, 19 bp, synthetic construct
  source 1..19: mol_type = other DNA
tccaaggaagatacacgcc

SEQ ID NO: 30 - DNA, 19 bp, synthetic construct
  source 1..19: mol_type = other DNA
ggtcgtagatttcatcggc

SEQ ID NO: 31 - DNA, 22 bp, synthetic construct
  source 1..22: mol_type = other DNA
caacggtgtctcagaactaatc

SEQ ID NO: 32 - DNA, 18 bp, synthetic construct
  source 1..18: mol_type = other DNA
tggtcgttggaatcttgc

SEQ ID NO: 33 - DNA, 57 bp, synthetic construct
  source 1..57: mol_type = other DNA
gcttgcatgcctgcaggtcgactctagaggatcccccaaagcacttgctactcaatc

SEQ ID NO: 34 - DNA, 56 bp, synthetic construct
  source 1..56: mol_type = other DNA
atcaggctgaaaatcttctctcatccgccaaaacctactgcttgtaagtggacagg

SEQ ID NO: 35 - DNA, 56 bp, synthetic construct
  source 1..56: mol_type = other DNA
cagtgccaagcttgcatgcctgcaggtcgactctaggcagcaagtagcctgggtat

SEQ ID NO: 36 - DNA, 35 bp, synthetic construct
  source 1..35: mol_type = other DNA
agaagatgaaggacgtgggtaacttcctgtccact

SEQ ID NO: 37 - DNA, 40 bp, synthetic construct
  source 1..40: mol_type = other DNA
agtggacaggaagttacccacgtccttcatcttctccgac

SEQ ID NO: 38 - DNA, 57 bp, synthetic construct
  source 1..57: mol_type = other DNA
cagctatgaccatgattacgaattcgagctcggtacccacgcaacacttgatggagt